European Patent Specification EP 3 613 858 B1, published March 13, 2024. Title: RECOMBINANT CORYNEBACTERIUM GLUTAMICUM FOR THE PRODUCTION OF 3'-FUCOSYLLACTOSE AND METHOD FOR THE PRODUCTION OF 3'-FUCOSYLLACTOSE THEREFROM. Applicant: Seoul National University R&DB Foundation. The sequence listing filed with the application follows.

SEQUENCE LISTING (7 sequences)

SEQ ID NO: 1 - DNA, 1377 bp, Unknown
  Corynebacterium glutamicum ATCC 13032
atgcgtacccgtgaatctgtcacggctgtaattaaggcgtatgacgtccgtggtgttgttggtgtcgatattgatgctgatttcatttctgagactggcgctgcctttggtcggctcatgcgtagtgagggtgaaaccaccgttgctattggccatgacatgcgtgattcctcccctgaattggccaaggcgtttgccgatggcgtgactgcacagggtttggatgttgttcatttgggactgacttctactgatgagctgtactttgcgtccggaaccttgaagtgtgctggtgcgatgtttactgcgtcgcataaccccgctgagtacaacggcatcaagttgtgtcgtgcgggtgctcgtccggtcggtcaggattctggtttggccaacatcattgatgatctggttgagggtgttccagcgtttgatggtgagtcaggttcggtttctgagcaggatttgctgagcgcatatgccgagtacctcaatgagcttgttgatctgaagaacatccgcccgttgaaggttgctgtggatgcggcaaacggcatgggtgggttcactgtccctgaggtattcaagggtctgccacttgatgttgcgccactgtattttgagcttgacggcaatttccccaaccatgaggccaatcctctggagcctgccaacctggttgatttgcagaagtttaccgtagagaccggatctgatatcggtttggcgttcgacggcgatgcggatcgttgcttcgtggtcgatgagaagggccagccagtcagcccttcggcgatctgtgcgatcgtagcggagcgttacttggagaagcttccgggttccaccatcatccacaacctgattacctctaaggctgtgcctgaggtgattgctgaaaacggtggcactgcggtgcgtactcgcgtgggtcactccttcatcaaggcgaagatggcagagaccggtgcggcctttggtggcgagcactctgcgcactactacttcactgagttcttcaatgcggactccggcattttggctgcgatgcacgtgctggctgcgctgggaagccaggaccagccactcagtgagatgatggctaggtataaccggtacgttgcttcaggcgagttgaactcccgtttggctaatgcagaggcgcagcaagagcgcacccaggctgtgctcgatgcgttcgctgatcgcaccgagtccgtggacacccttgacggcgtgactgtggaactcaaggacacctccgcgtggttcaacgtgcgtgcgtccaacaccgagccgctgcttcgcctcaatgttgaagctgcatcgaaggaagaagtcgatgcgttggtagcggagattctagggattatccgcgcataa

SEQ ID NO: 2 - DNA, 1089 bp, Unknown
  Corynebacterium glutamicum ATCC 13032
atgactttaactgacaacagcaaaaacgttgatgctgtcatcttggtcggtggcaaaggtacccgactgcgccccctgaccgtcaatactccaaagccaatgctgccaactgctggccacccattcttgacccaccttttggcccgcatcaaggccgcaggcatcacacacgtcgtgctgggaacgtcattcaaagctgaagtcttcgaggaatacttcggagatggctccgaaatgggcttggaaattgaatatgtcgtcgaggatcagcctttgggcactggtggtggcatccgaaacgtctacgacaagctgcgtcacgatactgcgattgtgttcaacggcgatgtgctctccggtgcggatctcaacagcattctggacacccaccgcgaaaaggacgcagatctgaccatgcatctcgtgcgcgtagctaaccctcgtgcgtttggttgcgtccccaccgatgaggatggtcgcgtcagcgaattccttgaaaagaccgaagatccaccaaccgatcagatcaacgccggctgctacgtgttcaagaaggaactcatcgagcagatcccggcaggccgagcagtttccgtcgagcgcgaaaccttccctcagctgttggaagaaggcaagcgagtcttcggccacgtcgacgcttcctactggcgcgacatgggcaccccaagcgacttcgtccgcggctcggctgacctggtccgcggcattgcgtactccccattgctcgaaggcaaaacaggagagtcgcttgtcgacgcctccgccggcgttcgcgacggcgtcctgctgctcggcggaaccgtagtcggccgcggcactgagatcggtgccggctgccgcgttgacaacactgttattttcgacggcgtcaccattgaaccaggtgcggtcattgaaaattccatcatttcctcgggagcacgcatcggtgctaatgcgcacatctccggttgcatcattggcgagggcgcacaggttggtgctcggtgtgaactcaacgcagggatgcgcgtcttcccaggcgttgtgatcccagacagcggaattcgtttttcgtctgatcagtag

SEQ ID NO: 3 - DNA, 2090 bp, Unknown
  E.coli K-12 MG1655
atgtcaaaagtcgctctcatcaccggtgtaaccggacaagacggttcttacctggcagagtttctgctggaaaaaggttacgaggtgcatggtattaagcgtcgcgcatcgtcattcaacaccgagcgcgtggatcacatttatcaggatccgcacacctgcaacccgaaattccatctgcattatggcgacctgagtgatacctctaacctgacgcgcattttgcgtgaagtacagccggatgaagtgtacaacctgggcgcaatgagccacgttgcggtctcttttgagtcaccagaatataccgctgacgtcgacgcgatgggtacgctgcgcctgctggaggcgatccgcttcctcggtctggaaaagaaaactcgtttctatcaggcttccacctctgaactgtatggtctggtgcaggaaattccgcagaaagagaccacgccgttctacccgcgatctccgtatgcggtcgccaaactgtacgcctactggatcaccgttaactaccgtgaatcctacggcatgtacgcctgtaacggaattctcttcaaccatgaatccccgcgccgcggcgaaaccttcgttacccgcaaaatcacccgcgcaatcgccaacatcgcccaggggctggagtcgtgcctgtacctcggcaatatggattccctgcgtgactggggccacgccaaagactacgtaaaaatgcagtggatgatgctgcagcaggaacagccggaagatttcgttatcgcgaccggcgttcagtactccgtgcgtcagttcgtggaaatggcggcagcacagctgggcatcaaactgcgctttgaaggcacgggcgttgaagagaagggcattgtggtttccgtcaccgggcatgacgcgccgggcgttaaaccgggtgatgtgattatcgctgttgacccgcgttacttccgtccggctgaagttgaaacgctgctcggcgacccgaccaaagcgcacgaaaaactgggctggaaaccggaaatcaccctcagagagatggtgtctgaaatggtggctaatgacctcgaagcggcgaaaaaacactctctgctgaaatctcacggctacgacgtggcgatcgcgctggagtcataagcatgagtaaacaacgagtttttattgctggtcatcgcgggatggtcggttccgccatcaggcggcagctcgaacagcgcggtgatgtggaactggtattacgcacccgcgacgagctgaacctgctggacagccgcgccgtgcatgatttctttgccagcgaacgtattgaccaggtctatctggcggcggcgaaagtgggcggcattgttgccaacaacacctatccggcggatttcatctaccagaacatgatgattgagagcaacatcattcacgccgcgcatcagaacgacgtgaacaaactgctgtttctcggatcgtcctgcatctacccgaaactggcaaaacagccgatggcagaaagcgagttgttgcagggcacgctggagccgactaacgagccttatgctattgccaaaatcgccgggatcaaactgtgcgaatcatacaaccgccagtacggacgcgattaccgctcagtcatgccgaccaacctgtacgggccacacgacaacttccacccgagtaattcgcatgtgatcccagcattgctgcgtcgcttccacgaggcgacggcacagaatgcgccggacgtggtggtatggggcagcggtacaccgatgcgcgaatttctgcacgtcgatgatatggcggcggcgagcattcatgtcatggagctggcgcatgaagtctggctggagaacacccagccgatgttgtcgcacattaacgtcggcacgggcgttgactgcactatccgcgagctggcgcaaaccatcgccaaagtggtgggttacaaaggccgggtggtttttgatgccagcaaaccggatggcacgccgcgcaaactgctggatgtgacgcgcctgcatcagcttggctggtatcacgaaatctcactggaagcggggcttgccagcacttaccagtggttccttgagaatcaagaccgctttcgggggtaa

SEQ ID NO: 4 - DNA, 3335 bp, Unknown
  E.coli BL21star(DE3)
accatcgaatggcgcaaaacctttcgcggtatggcatgatagcgcccggaagagagtcaattcagggtggtgaatgtgaaaccagtaacgttatacgatgtcgcagagtatgccggtgtctcttatcagaccgtttcccgcgtggtgaaccaggccagccacgtttctgcgaaaacgcgggaaaaagtggaagcggcgatggcggagctgaattacattcccaaccgcgtggcacaacaactggcgggcaaacagtcgttgctgattggcgttgccacctccagtctggccctgcacgcgccgtcgcaaattgtcgcggcgattaaatctcgcgccgatcaactgggtgccagcgtggtggtgtcgatggtagaacgaagcggcgtcgaagcctgtaaagcggcggtgcacaatcttctcgcgcaacgcgtcagtgggctgatcattaactatccgctggatgaccaggatgccattgctgtggaagctgcctgcactaatgttccggcgttatttcttgatgtctctgaccagacacccatcaacagtattattttctcccatgaagacggtacgcgactgggcgtggagcatctggtcgcattgggtcaccagcaaatcgcgctgttagcgggcccattaagttctgtctcggcgcgtctgcgtctggctggctggcataaatatctcactcgcaatcaaattcagccgatagcggaacgggaaggcgactggagtgccatgtccggttttcaacaaaccatgcaaatgctgaatgagggcatcgttcccactgcgatgctggttgccaacgatcagatggcgctgggcgcaatgcgcgccattaccgagtccgggctgcgcgttggtgcggatatctcggtagtgggatacgacgataccgaagacagctcatgttatatcccgccgttaaccaccatcaaacaggattttcgcctgctggggcaaaccagcgtggaccgcttgctgcaactctctcagggccaggcggtgaagggcaatcagctgttgcccgtctcactggtgaaaagaaaaaccaccctggcgcccaatacgcaaaccgcctctccccgcgcgttggccgattcattaatgcagctggcacgacaggtttcccgactggaaagcgggcagtgagcgcaacgcaattaatgtgagttagctcactcattaggcaccccaggctttacactttatgcttccggctcgtatgttgtgtggaattgtgagcggataacaatttcacacaggaaacagctatgtactatttaaaaaacacaaacttttggatgttcggtttattctttttcttttacttttttatcatgggagcctacttcccgtttttcccgatttggctacatgacatcaaccatatcagcaaaagtgatacgggtattatttttgccgctatttctctgttctcgctattattccaaccgctgtttggtctgctttctgacaaactcgggctgcgcaaatacctgctgtggattattaccggcatgttagtgatgtttgcgccgttctttatttttatcttcgggccactgttacaatacaacattttagtaggatcgattgttggtggtatttatctaggcttttgttttaacgccggtgcgccagcagtagaggcatttattgagaaagtcagccgtcgcagtaatttcgaatttggtcgcgcgcggatgtttggctgtgttggctgggcgctgtgtgcctcgattgtcggcatcatgttcaccatcaataatcagtttgttttctggctgggctctggctgtgcactcatcctcgccgttttactctttttcgccaaaacggatgcgccctcttctgccacggttgccaatgcggtaggtgccaaccattcggcatttagccttaagctggcactggaactgttcagacagccaaaactgtggtttttgtcactgtatgttattggcgtttcctgcacctacgatgtttttgaccaacagtttgctaatttctttacttcgttctttgctaccggtgaacagggtacgcgggtatttggctacgtaacgacaatgggcgaattacttaacgcctcgattatgttctttgcgccactgatcattaatcgcatcggtgggaaaaacgccctgctgctggctggcactattatgtctgtacgtattattggctcatcgttcgccacctcagcgctggaagtggttattctgaaaacgctgcatatgtttgaagtaccgttcctgctggtgggctgctttaaatatattaccagccagtttgaagtgcgtttttcagcgacgatttatctggtctgtttctgcttctttaagcaactggcgatgatttttatgtctgtactggcgggcaatatgtatgaaagcatcggtttccagggcgcttatctggtgctgggtctggtggcgctgggcttcaccttaatttccgtgttcacgcttagcggccccggcccgctttccctgctgcgtcgtcaggtgaatgaagtcgcttaagcaatcaatgtcggatgcggcgcgagcgccttatccgaccaacatatcataacggagtgatcgcattgaacatgccaatgaccgaaagaataagagcaggcaagctatttaccgatatgtgcgaaggcttaccggaaaaaagacttcgtgggaaaacgttaatgtatgagtttaatcactcgcatccatcagaagttgaaaaaagagaaagcctgattaaagaaatgtttgccacggtaggggaaaacgcctgggtagaaccgcctgtctatttctcttacggttccaacatccatataggccgcaatttttatgcaaatttcaatttaaccattgtcgatgactacacggtaacaatcggtgataacgtactgattgcacccaacgttactctttccgttacgggacaccctgtacaccatgaattgagaaaaaacggcgagatgtactcttttccgataacgattggcaataacgtctggatcggaagtcatgtggttattaatccaggcgtcaccatcggggataattctgttattggcgcgggtagtatcgtcacaaaagacattccaccaaacgtcgtggcggctggcgttccttgtcgggttattcgcgaaataaacgaccgggataagcactattatttcaaagattataaagttgaatcgtcagtttaaattataaaaattgcctgatacgctgcgcttatcaggcctacaagttcagcgatctacattagccgcatccggcatgaacaaagcgcaggaacaagcgtcgcatcatgcctctttgacccacagc

SEQ ID NO: 5 - DNA, 978 bp, Unknown
  Azospirillum brasilense ATCC 29145
atgctcgatcagcggacaagcgcgtttcttgaggaattcctggcgaagccgggcggcgatcccgagcggctcgaccgcttcctgctgcacggcccgtaccgcggccggcgcggcggcaaaccgcggctgaagctggccttccacgacttctggccggagttcgacaagggcacgaacttcttcatcgagatcctgtccagccgcttcgacctgtcggtggtcgaggacgacagcgacctcgccatcgtgtcggtcttcggcgggcggcaccgcgaggcgcgcagccgccgcaccctgttcttcaccggggagaacgtgcgcccgccgttggacggcttcgacatggcggtgtccttcgaccgcgtcgacgacccgcgccattaccgcctgccgctctacgtcatgcacgcctacgagcacatgcgggagggggcggtgccgcatttctgttcgccggtcctgccgccggtgccgccgacgcgggcggccttcgcggagcgcggcttctgcgccttcctctacaagaacccgaacggggagcgccgcaaccgcttcttcccggtgctggacgggcggcggcgcgtcgattcggtgggctggcacctgaacaacaccggcagcgtcgtcaagatgggctggctgtcgaagatccgcgtcttcgaacgctaccgtttcgccttcgccttcgagaacgccagccatcccggctatctgacggaaaagatcctggacgtcttccaggccggggcggtgccgctctattggggtgatcccgacctggagcgcgaggtggcggtcggcagcttcatcgacgtgtcgcgcttcgccacggacgaggaggcggtggaccacatccttgcggtggacgacgattacgacgcctattgcgcccaccgcgccgtggcgcccttcctggggacggaggagttttatttcgacgcctaccgcctcgccgactggatcgagagccggctgtaa

SEQ ID NO: 6 - DNA, 54 bp, Artificial Sequence
  F_inf_sac1_azoT
gctttcgggggtaagagctcaaggagatatacaatgctcgatcagcggacaagc

SEQ ID NO: 7 - DNA, 40 bp, Artificial Sequence
  R_inf_sac1_azoT
cggccagtgaattcgagctcttacagccggctctcgatcc